European Patent Application EP 4 249 497 A1, published September 27, 2023. Title: Novel SST4 selective agonists as non-opioid analgesics. Applicant: University of Copenhagen. The sequence listing filed with the application follows.

SEQUENCE LISTING (14 sequences)

SEQ ID NO: 1 - protein, 10 aa, Cone snail
  HSH-109
PVCWKFGCPL

SEQ ID NO: 2 - protein, 9 aa, Cone snail
  HSH-133
LFCWKFGCW

SEQ ID NO: 3 - protein, 9 aa, Cone snail
  HSH-142
PVCWKFGCW

SEQ ID NO: 4 - protein, 10 aa, Cone snail
  HSH-153
PVCWKFACPL

SEQ ID NO: 5 - protein, 10 aa, Cone snail
  HSH-141
LFCWKFGCPL

SEQ ID NO: 6 - protein, 9 aa, Cone snail
  HSH-149
PVCWKFCPL

SEQ ID NO: 7 - protein, 10 aa, Cone snail
  HSH-147
PVCWKFGCPL

SEQ ID NO: 8 - protein, 10 aa, Cone snail
  HSH-143
PVCWKFGCPL

SEQ ID NO: 9 - protein, 10 aa, Cone snail
  HSH-148
PVCWKFGCPL

SEQ ID NO: 10 - protein, 8 aa, Cone snail
  HSH-146
PVCWKFGC

SEQ ID NO: 11 - protein, 6 aa, Cone snail
  HSH-144
CWKFGC

SEQ ID NO: 12 - protein, 8 aa, Cone snail
  HSH-145
CWKFGCPL

SEQ ID NO: 13 - protein, 10 aa, Cone snail
  HSH-152
PVCWKAGCPL

SEQ ID NO: 14 - protein, 10 aa, Cone snail
  HSH-151
PVCWAFGCPL